European Patent Application EP 4 582 106 A1, published July 9, 2025. Title: ANTIBODY-DRUG CONJUGATE INCLUDING MUTANT FC REGION. Applicant: DAIICHI SANKYO COMPANY, LIMITED. Application EP 23860252.8, filed August 28, 2023. The sequence listing filed with the application follows.

SEQUENCE LISTING (56 sequences)

SEQ ID NO: 1 - protein, 379 aa, Homo sapiens [sequence omitted]

SEQ ID NO: 2 - DNA, 1140 bp, Homo sapiens
  source 1..1140: mol_type = genomic DNA
atgccccactccagcctgcatccatccatcccgtgtcccaggggtcacggggcccagaaggcagccttggttctgctgagtgcctgcctggtgaccctttgggggctaggagagccaccagagcacactctccggtacctggtgctccacctagcctccctgcagctgggactgctgttaaacggggtctgcagcctggctgaggagctgcgccacatccactccaggtaccggggcagctactggaggactgtgcgggcctgcctgggctgccccctccgccgtggggccctgttgctgctgtccatctatttctactactccctcccaaatgcggtcggcccgcccttcacttggatgcttgccctcctgggcctctcgcaggcactgaacatcctcctgggcctcaagggcctggccccagctgagatctctgcagtgtgtgaaaaagggaatttcaacgtggcccatgggctggcatggtcatattacatcggatatctgcggctgatcctgccagagctccaggcccggattcgaacttacaatcagcattacaacaacctgctacggggtgcagtgagccagcggctgtatattctcctcccattggactgtggggtgcctgataacctgagtatggctgaccccaacattcgcttcctggataaactgccccagcagaccggtgaccatgctggcatcaaggatcgggtttacagcaacagcatctatgagcttctggagaacgggcagcgggcgggcacctgtgtcctggagtacgccacccccttgcagactttgtttgccatgtcacaatacagtcaagctggctttagccgggaggataggcttgagcaggccaaactcttctgccggacacttgaggacatcctggcagatgcccctgagtctcagaacaactgccgcctcattgcctaccaggaacctgcagatgacagcagcttctcgctgtcccaggaggttctccggcacctgcggcaggaggaaaaggaagaggttactgtgggcagcttgaagacctcagcggtgcccagtacctccacgatgtcccaagagcctgagctcctcatcagtggaatggaaaagcccctccctctccgcacggatttctcttag

SEQ ID NO: 3 - protein, 379 aa, Homo sapiens
MPHSSLHPSIPCPRGHGAQKAALVLLSACLVTLWGLGEPPEHTLRYLVLHLASLQLGLLLNGVCSLAEELRHIHSRYRGSYWRTVRACLGCPLRRGALLLLSIYFYYSLPNAVGPPFTWMLALLGLSQALNILLGLKGLAPAEISAVCEKGNFNVAHGLAWSYYIGYLRLILPELQARIRTYNQHYNNLLRGAVSQRLYILLPLDCGVPDNLSMADPNIRFLDKLPQQTGDHAGIKDRVYSNSIYELLENGQRAGTCVLEYATPLQTLFAMSQYSQAGFSREDRLEQAKLFCRTLEDILADAPESQNNCRLIAYQEPADDSSFSLSQEVLRHLRQEEKEEVTVGSLKTSAVPSTSTMSQEPELLISGMEKPLPLRTDFS

SEQ ID NO: 4 - DNA, 1140 bp, Homo sapiens
  source 1..1140: mol_type = genomic DNA
  misc_difference 1..1140
atgccccactccagcctgcatccatccatcccgtgtcccaggggtcacggggcccagaaggcagccttggttctgctgagtgcctgcctggtgaccctttgggggctaggagagccaccagagcacactctccggtacctggtgctccacctagcctccctgcagctgggactgctgttaaacggggtctgcagcctggctgaggagctgcgccacatccactccaggtaccggggcagctactggaggactgtgcgggcctgcctgggctgccccctccgccgtggggccctgttgctgctgtccatctatttctactactccctcccaaatgcggtcggcccgcccttcacttggatgcttgccctcctgggcctctcgcaggcactgaacatcctcctgggcctcaagggcctggccccagctgagatctctgcagtgtgtgaaaaagggaatttcaacgtggcccatgggctggcatggtcatattacatcggatatctgcggctgatcctgccagagctccaggcccggattcgaacttacaatcagcattacaacaacctgctacggggtgcagtgagccagcggctgtatattctcctcccattggactgtggggtgcctgataacctgagtatggctgaccccaacattcgcttcctggataaactgccccagcagaccggtgaccgtgctggcatcaaggatcgggtttacagcaacagcatctatgagcttctggagaacgggcagcgggcgggcacctgtgtcctggagtacgccacccccttgcagactttgtttgccatgtcacaatacagtcaagctggctttagccgggaggataggcttgagcaggccaaactcttctgccggacacttgaggacatcctggcagatgcccctgagtctcagaacaactgccgcctcattgcctaccaggaacctgcagatgacagcagcttctcgctgtcccaggaggttctccggcacctgcggcaggaggaaaaggaagaggttactgtgggcagcttgaagacctcagcggtgcccagtacctccacgatgtcccaagagcctgagctcctcatcagtggaatggaaaagcccctccctctccgcacggatttctcttag

SEQ ID NO: 5 - protein, 379 aa, Homo sapiens
MPHSSLHPSIPCPRGHGAQKAALVLLSACLVTLWGLGEPPEHTLRYLVLHLASLQLGLLLNGVCSLAEELHHIHSRYRGSYWRTVRACLGCPLRRGALLLLSIYFYYSLPNAVGPPFTWMLALLGLSQALNILLGLKGLAPAEISAVCEKGNFNVAHGLAWSYYIGYLRLILPELQARIRTYNQHYNNLLRGAVSQRLYILLPLDCGVPDNLSMADPNIRFLDKLPQQTADRAGIKDRVYSNSIYELLENGQRAGTCVLEYATPLQTLFAMSQYSQAGFSREDRLEQAKLFCQTLEDILADAPESQNNCRLIAYQEPADDSSFSLSQEVLRHLRQEEKEEVTVGSLKTSAVPSTSTMSQEPELLISGMEKPLPLRTDFS

SEQ ID NO: 6 - DNA, 1140 bp, Homo sapiens
  source 1..1140: mol_type = other DNA
  misc_difference 1..1140
atgccccactccagcctgcatccatccatcccgtgtcccaggggtcacggggcccagaaggcagccttggttctgctgagtgcctgcctggtgaccctttgggggctaggagagccaccagagcacactctccggtacctggtgctccacctagcctccctgcagctgggactgctgttaaacggggtctgcagcctggctgaggagctgcaccacatccactccaggtaccggggcagctactggaggactgtgcgggcctgcctgggctgccccctccgccgtggggccctgttgctgctgtccatctatttctactactccctcccaaatgcggtcggcccgcccttcacttggatgcttgccctcctgggcctctcgcaggcactgaacatcctcctgggcctcaagggcctggccccagctgagatctctgcagtgtgtgaaaaagggaatttcaacgtggcccatgggctggcatggtcatattacatcggatatctgcggctgatcctgccagagctccaggcccggattcgaacttacaatcagcattacaacaacctgctacggggtgcagtgagccagcggctgtatattctcctcccattggactgtggggtgcctgataacctgagtatggctgaccccaacattcgcttcctggataaactgccccagcagaccgctgaccgtgctggcatcaaggatcgggtttacagcaacagcatctatgagcttctggagaacgggcagcgggcgggcacctgtgtcctggagtacgccacccccttgcagactttgtttgccatgtcacaatacagtcaagctggctttagccgggaggataggcttgagcaggccaaactcttctgccagacacttgaggacatcctggcagatgcccctgagtctcagaacaactgccgcctcattgcctaccaggaacctgcagatgacagcagcttctcgctgtcccaggaggttctccggcacctgcggcaggaggaaaaggaagaggttactgtgggcagcttgaagacctcagcggtgcccagtacctccacgatgtcccaagagcctgagctcctcatcagtggaatggaaaagcccctccctctccgcacggatttctcttag

SEQ ID NO: 7 - protein, 378 aa, Mus musculus
MPYSNLHPAIPRPRGHRSKYVALIFLVASLMILWVAKDPPNHTLKYLALHLASHELGLLLKNLCCLAEELCHVQSRYQGSYWKAVRACLGCPIHCMAMILLSSYFYFLQNTADIYLSWMFGLLVLYKSLSMLLGLQSLTPAEVSAVCEEKKLNVAHGLAWSYYIGYLRLILPGLQARIRMFNQLHNNMLSGAGSRRLYILFPLDCGVPDNLSVVDPNIRFRDMLPQQNIDRAGIKNRVYSNSVYEILENGQPAGVCILEYATPLQTLFAMSQDAKAGFSREDRLEQAKLFCRTLEEILEDVPESRNNCRLIVYQEPTDGNSFSLSQEVLRHIRQEEKEEVTMNAPMTSVAPPPSVLSQEPRLLISGMDQPLPLRTDLI

SEQ ID NO: 8 - DNA, 1137 bp, Mus musculus
  source 1..1137: mol_type = genomic DNA
atgccatactccaacctgcatccagccatcccacggcccagaggtcaccgctccaaatatgtagccctcatctttctggtggccagcctgatgatcctttgggtggcaaaggatccaccaaatcacactctgaagtacctagcacttcacctagcctcgcacgaacttggactactgttgaaaaacctctgctgtctggctgaagagctgtgccatgtccagtccaggtaccagggcagctactggaaggctgtgcgcgcctgcctgggatgccccatccactgtatggctatgattctactatcgtcttatttctatttcctccaaaacactgctgacatatacctcagttggatgtttggccttctggtcctctataagtccctaagcatgctcctgggccttcagagcttgactccagcggaagtctctgcagtctgtgaagaaaagaagttaaatgttgcccacgggctggcctggtcatactacattgggtacttgcggttgatcttaccagggctccaggcccggatccgaatgttcaatcagctacataacaacatgctcagtggtgcagggagccgaagactgtacatcctctttccattggactgtggggtgcctgacaacctgagtgtagttgaccccaacattcgattccgagatatgctgccccagcaaaacatcgaccgtgctggcatcaagaatcgggtttattccaacagcgtctacgagattctggagaacggacagccagcaggcgtctgtatcctggagtacgccacccccttgcagaccctgtttgccatgtcacaggatgccaaagctggcttcagtcgggaggatcggcttgagcaggctaaactcttctgccggacacttgaggaaatcctggaagatgtccccgagtctcgaaataactgccgcctcattgtctaccaagaacccacagacggaaacagtttctcactgtctcaggaggtgctccggcacattcgtcaggaagaaaaggaggaggttaccatgaatgcccccatgacctcagtggcacctcctccctccgtactgtcccaagagccaagactcctcatcagtggtatggatcagcctctcccactccgcactgacctcatctga

SEQ ID NO: 9 - protein, 243 aa, Homo sapiens
MGSSHHHHHHSSGSGLNDIFEAQKIEWHEGGSENLYFQGLAPAEISAVCEKGNFNVAHGLAWSYYIGYLRLILPELQARIRTYNQHYNNLLRGAVSQRLYILLPLDCGVPDNLSMADPNIRFLDKLPQQTGDRAGIKDRVYSNSIYELLENGQRAGTCVLEYATPLQTLFAMSQYSQAGFSREDRLEQAKLFCRTLEDILADAPESQNNCRLIAYQEPADDSSFSLSQEVLRHLRQEEKEEVT

SEQ ID NO: 10 - protein, 243 aa, Homo sapiens
MGSSHHHHHHSSGSGLNDIFEAQKIEWHEGGSENLYFQGLAPAEISAVCEKGNFNVAHGLAWSYYIGYLRLILPELQARIRTYNQHYNNLLRGAVSQRLYILLPLDCGVPDNLSMADPNIRFLDKLPQQTGDHAGIKDRVYSNSIYELLENGQRAGTCVLEYATPLQTLFAMSQYSQAGFSREDRLEQAKLFCRTLEDILADAPESQNNCRLIAYQEPADDSSFSLSQEVLRHLRQEEKEEVT

SEQ ID NO: 11 - protein, 243 aa, Homo sapiens
MGSSHHHHHHSSGSGLNDIFEAQKIEWHEGGSENLYFQGLAPAEISAVCEKGNFNVAHGLAWSYYIGYLRLILPELQARIRTYNQHYNNLLRGAVSQRLYILLPLDCGVPDNLSMADPNIRFLDKLPQQTADRAGIKDRVYSNSIYELLENGQRAGTCVLEYATPLQTLFAMSQYSQAGFSREDRLEQAKLFCQTLEDILADAPESQNNCRLIAYQEPADDSSFSLSQEVLRHLRQEEKEEVT

SEQ ID NO: 12 - protein, 243 aa, Mus musculus
MGSSHHHHHHSSGSGLNDIFEAQKIEWHEGGSENLYFQGLTPAEVSAVCEEKKLNVAHGLAWSYYIGYLRLILPGLQARIRMFNQLHNNMLSGAGSRRLYILFPLDCGVPDNLSVVDPNIRFRDMLPQQNIDRAGIKNRVYSNSVYEILENGQPAGVCILEYATPLQTLFAMSQDAKAGFSREDRLEQAKLFCRTLEEILEDVPESRNNCRLIVYQEPTDGNSFSLSQEVLRHIRQEEKEEVT

SEQ ID NO: 13 - DNA, 27 bp, synthetic construct
  misc_feature 1..27: note = primer
  source 1..27: mol_type = other DNA
cgtgctggcatcaaggatcgggtttac

SEQ ID NO: 14 - DNA, 27 bp, synthetic construct
  misc_feature 1..27: note = primer
  source 1..27: mol_type = other DNA
gtcaccggtctgctggggcagtttatc

SEQ ID NO: 15 - DNA, 33 bp, synthetic construct
  misc_feature 1..33: note = primer
  source 1..33: mol_type = other DNA
gctgaccgtgctggcatcaaggatcgggtttac

SEQ ID NO: 16 - DNA, 25 bp, synthetic construct
  misc_feature 1..25: note = primer
  source 1..25: mol_type = other DNA
ggtctgctggggcagtttatccagg

SEQ ID NO: 17 - DNA, 24 bp, synthetic construct
  misc_feature 1..24: note = primer
  source 1..24: mol_type = other DNA
caccacatccactccaggtaccgg

SEQ ID NO: 18 - DNA, 24 bp, synthetic construct
  misc_feature 1..24: note = primer
  source 1..24: mol_type = other DNA
cagctcctcagccaggctgcagac

SEQ ID NO: 19 - DNA, 25 bp, synthetic construct
  misc_feature 1..25: note = primer
  source 1..25: mol_type = other DNA
cagacacttgaggacatcctggcag

SEQ ID NO: 20 - DNA, 23 bp, synthetic construct
  misc_feature 1..23: note = primer
  source 1..23: mol_type = other DNA
gcagaagagtttggcctgctcaa

SEQ ID NO: 21 - DNA, 39 bp, synthetic construct
  misc_feature 1..39: note = primer
  source 1..39: mol_type = other DNA
acctgtattttcagggcctggccccagctgagatctctg

SEQ ID NO: 22 - DNA, 44 bp, synthetic construct
  misc_feature 1..44: note = primer
  source 1..44: mol_type = other DNA
cagaattcgcaagcttttaagtaacctcttccttttcctcctgc

SEQ ID NO: 23 - protein, 11 aa, Homo sapiens
QASQDISNYLN

SEQ ID NO: 24 - protein, 7 aa, Homo sapiens
DASNLET

SEQ ID NO: 25 - protein, 9 aa, Homo sapiens
QHFDHLPLA

SEQ ID NO: 26 - protein, 7 aa, Homo sapiens
SGDYYWT

SEQ ID NO: 27 - protein, 16 aa, Homo sapiens
HIYYSGNTNYNPSLKS

SEQ ID NO: 28 - protein, 9 aa, Homo sapiens
DRVTGAFDI

SEQ ID NO: 29 - protein, 108 aa, Homo sapiens
DIQMTQSPSSLSASVGDRVTITCQASQDISNYLNWYQQKPGKAPKLLIYDASNLETGVPSRFSGSGSGTDFTFTISSLQPEDIATYFCQHFDHLPLAFGGGTKVEIKR

SEQ ID NO: 30 - protein, 214 aa, Homo sapiens
DIQMTQSPSSLSASVGDRVTITCQASQDISNYLNWYQQKPGKAPKLLIYDASNLETGVPSRFSGSGSGTDFTFTISSLQPEDIATYFCQHFDHLPLAFGGGTKVEIKRTVAAPSVFIFPPSDEQLKSGTASVVCLLNNFYPREAKVQWKVDNALQSGNSQESVTEQDSKDSTYSLSSTLTLSKADYEKHKVYACEVTHQGLSSPVTKSFNRGEC

SEQ ID NO: 31 - protein, 119 aa, Homo sapiens [sequence omitted]

SEQ ID NO: 32 - protein, 449 aa, Homo sapiens
QVQLQESGPGLVKPSETLSLTCTVSGGSVSSGDYYWTWIRQSPGKGLEWIGHIYYSGNTNYNPSLKSRLTISIDTSKTQFSLKLSSVTAADTAIYYCVRDRVTGAFDIWGQGTMVTVSSASTKGPSVFPLAPSSKSTSGGTAALGCLVKDYFPEPVTVSWNSGALTSGVHTFPAVLQSSGLYSLSSVVTVPSSSLGTQTYICNVNHKPSNTKVDKRVEPKSCDKTHTCPPCPAPEAAGGPSVFLFPPKPKDTLMISRTPEVTCVVVGVSHEDPEVKFNWYVDGVEVHNAKTKPREEQYNSTYRVVSVLTVLHQDWLNGKEYKCKVSNKALPAPIEKTISKAKGQPREPQVYTLPPSREEMTKNQVSLTCLVKGFYPSDIAVEWESNGQPENNYKTTPPVLDSDGSFFLYSKLTVDKSRWQQGNVFSCSVMHEALHNHYTQKSLSLSPGK

SEQ ID NO: 33 - protein, 449 aa, Homo sapiens
QVQLQESGPGLVKPSETLSLTCTVSGGSVSSGDYYWTWIRQSPGKGLEWIGHIYYSGNTNYNPSLKSRLTISIDTSKTQFSLKLSSVTAADTAIYYCVRDRVTGAFDIWGQGTMVTVSSASTKGPSVFPLAPSSKSTSGGTAALGCLVKDYFPEPVTVSWNSGALTSGVHTFPAVLQSSGLYSLSSVVTVPSSSLGTQTYICNVNHKPSNTKVDKKVEPKSCDKTHTCPPCPAPEAAGGPSVFLFPPKPKDTLMISRTPEVTCVVVGVSHEDPEVKFNWYVDGVEVHNAKTKPREEQYNSTYRVVSVLTVLHQDWLNGKEYKCKVSNKALPAPIEKTISKAKGQPREPQVYTLPPSREEMTKNQVSLTCLVKGFYPSDIAVEWESNGQPENNYKTTPPVLDSDGSFFLYSKLTVDKSRWQQGNVFSCSVMHEALHNHYTQKSLSLSPGK

SEQ ID NO: 34 - protein, 449 aa, Homo sapiens
QVQLQESGPGLVKPSETLSLTCTVSGGSVSSGDYYWTWIRQSPGKGLEWIGHIYYSGNTNYNPSLKSRLTISIDTSKTQFSLKLSSVTAADTAIYYCVRDRVTGAFDIWGQGTMVTVSSASTKGPSVFPLAPSSKSTSGGTAALGCLVKDYFPEPVTVSWNSGALTSGVHTFPAVLQSSGLYSLSSVVTVPSSSLGTQTYICNVNHKPSNTKVDKRVEPKSCDKTHTCPPCPAPELLGGPSVFLFPPKPKDTLMISRTPEVTCVVVDVSHEDPEVKFNWYVDGVEVHNAKTKPREEQYNSTYRVVSVLTVLHQDWLNGKEYKCKVSNKALPAPIEKTISKAKGQPREPQVYTLPPSREEMTKNQVSLTCLVKGFYPSDIAVEWESNGQPENNYKTTPPVLDSDGSFFLYSKLTVDKSRWQQGNVFSCSVMHEALHNHYTQKSLSLSPGK

SEQ ID NO: 35 - protein, 445 aa, Homo sapiens
QVQLQESGPGLVKPSETLSLTCTVSGGSVSSGDYYWTWIRQSPGKGLEWIGHIYYSGNTNYNPSLKSRLTISIDTSKTQFSLKLSSVTAADTAIYYCVRDRVTGAFDIWGQGTMVTVSSASTKGPSVFPLAPCSRSTSESTAALGCLVKDYFPEPVTVSWNSGALTSGVHTFPAVLQSSGLYSLSSVVTVPSSNFGTQTYTCNVDHKPSNTKVDKTVERKCCVECPPCPAPPVAGPSVFLFPPKPKDTLMISRTPEVTCVVVDVSHEDPEVQFNWYVDGVEVHNAKTKPREEQFNSTFRVVSVLTVVHQDWLNGKEYKCKVSNKGLPAPIEKTISKTKGQPREPQVYTLPPSREEMTKNQVSLTCLVKGFYPSDIAVEWESNGQPENNYKTTPPMLDSDGSFFLYSKLTVDKSRWQQGNVFSCSVMHEALHNHYTQKSLSLSPGK

SEQ ID NO: 36 - protein, 449 aa, Homo sapiens
QVQLQESGPGLVKPSETLSLTCTVSGGSVSSGDYYWTWIRQSPGKGLEWIGHIYYSGNTNYNPSLKSRLTISIDTSKTQFSLKLSSVTAADTAIYYCVRDRVTGAFDIWGQGTMVTVSSASTKGPSVFPLAPSSKSTSGGTAALGCLVKDYFPEPVTVSWNSGALTSGVHTFPAVLQSSGLYSLSSVVTVPSSSLGTQTYICNVNHKPSNTKVDKRVEPKSCDKTHTCPPCPAPEAAGGPSVFLFPPKPKDTLMISRTPEVTCVVVDVSHEDPEVKFNWYVDGVEVHNAKTKPREEQYNSTYRVVSVLTVLHQDWLNGKEYKCKVSNKALPAPIEKTISKAKGQPREPQVYTLPPSREEMTKNQVSLTCLVKGFYPSDIAVEWESNGQPENNYKTTPPVLDSDGSFFLYSKLTVDKSRWQQGNVFSCSVMHEALHNHYTQKSLSLSPGK

SEQ ID NO: 37 - protein, 11 aa, Homo sapiens
KASQNIYKNLA

SEQ ID NO: 38 - protein, 7 aa, Homo sapiens
DANTLQT

SEQ ID NO: 39 - protein, 8 aa, Homo sapiens
QQYYSGWA

SEQ ID NO: 40 - protein, 5 aa, Homo sapiens
RNFMH

SEQ ID NO: 41 - protein, 17 aa, Homo sapiens
WIYPGDGETEYAQKFQG

SEQ ID NO: 42 - protein, 13 aa, Homo sapiens
GVYGGFAGGYFDF

SEQ ID NO: 43 - protein, 107 aa, Homo sapiens
DIQMTQSPSSLSASVGDRVTITCKASQNIYKNLAWYQQKPGKAPKLLIYDANTLQTGVPSRFSGSGSGSDFTLTISSLQPEDFATYFCQQYYSGWAFGQGTKVEIKR

SEQ ID NO: 44 - protein, 213 aa, Homo sapiens
DIQMTQSPSSLSASVGDRVTITCKASQNIYKNLAWYQQKPGKAPKLLIYDANTLQTGVPSRFSGSGSGSDFTLTISSLQPEDFATYFCQQYYSGWAFGQGTKVEIKRTVAAPSVFIFPPSDEQLKSGTASVVCLLNNFYPREAKVQWKVDNALQSGNSQESVTEQDSKDSTYSLSSTLTLSKADYEKHKVYACEVTHQGLSSPVTKSFNRGEC

SEQ ID NO: 45 - protein, 122 aa, Homo sapiens
EVQLVQSGAEVKKPGASVKVSCKASGYTFTRNFMHWVRQAPGQGLEWMGWIYPGDGETEYAQKFQGRVTITADTSTSTAYMELSSLRSEDTAVYYCARGVYGGFAGGYFDFWGQGTLVTVSS

SEQ ID NO: 46 - protein, 452 aa, Homo sapiens
EVQLVQSGAEVKKPGASVKVSCKASGYTFTRNFMHWVRQAPGQGLEWMGWIYPGDGETEYAQKFQGRVTITADTSTSTAYMELSSLRSEDTAVYYCARGVYGGFAGGYFDFWGQGTLVTVSSASTKGPSVFPLAPSSKSTSGGTAALGCLVKDYFPEPVTVSWNSGALTSGVHTFPAVLQSSGLYSLSSVVTVPSSSLGTQTYICNVNHKPSNTKVDKKVEPKSCDKTHTCPPCPAPEAAGGPSVFLFPPKPKDTLMISRTPEVTCVVVGVSHEDPEVKFNWYVDGVEVHNAKTKPREEQYNSTYRVVSVLTVLHQDWLNGKEYKCKVSNKALPAPIEKTISKAKGQPREPQVYTLPPSREEMTKNQVSLTCLVKGFYPSDIAVEWESNGQPENNYKTTPPVLDSDGSFFLYSKLTVDKSRWQQGNVFSCSVMHEALHNHYTQKSLSLSPGK

SEQ ID NO: 47 - protein, 995 aa, Streptococcus pyogenes
MDKHLLVKRTLGCVCAATLMGAALATHHDSLNTVKAEEKTVQVQKGLPSIDSLHYLSENSKKEFKEELSKAGQESQKVKEILAKAQQADKQAQELAKMKIPEKIPMKPLHGPLYGGYFRTWHDKTSDPTEKDKVNSMGELPKEVDLAFIFHDWTKDYSLFWKELATKHVPKLNKQGTRVIRTIPWRFLAGGDNSGIAEDTSKYPNTPEGNKALAKAIVDEYVYKYNLDGLDVDVEHDSIPKVDKKEDTAGVERSIQVFEEIGKLIGPKGVDKSRLFIMDSTYMADKNPLIERGAPYINLLLVQVYGSQGEKGGWEPVSNRPEKTMEERWQGYSKYIRPEQYMIGFSFYEENAQEGNLWYDINSRKDEDKANGINTDITGTRAERYARWQPKTGGVKGGIFSYAIDRDGVAHQPKKYAKQKEFKDATDNIFHSDYSVSKALKTVMLKDKSYDLIDEKDFPDKALREAVMAQVGTRKGDLERFNGTLRLDNPAIQSLEGLNKFKKLAQLDLIGLSRITKLDRSVLPANMKPGKDTLETVLETYKKDNKEEPATIPPVSLKVSGLTGLKELDLSGFDRETLAGLDAATLTSLEKVDISGNKLDLAPGTENRQIFDTMLSTISNHVGSNEQTVKFDKQKPTGHYPDTYGKTSLRLPVANEKVDLQSQLLFGTVTNQGTLINSEADYKAYQNHKIAGRSFVDSNYHYNNFKVSYENYTVKVTDSTLGTTTDKTLATDKEETYKVDFFSPADKTKAVHTAKVIVGDEKTMMVNLAEGATVIGGSADPVNARKVFDGQLGSETDNISLGWDSKQSIIFKLKEDGLIKHWRFFNDSARNPETTNKPIQEASLQIFNIKDYNLDNLLENPNKFDDEKYWITVDTYSAQGERATAFSNTLNNITSKYWRVVFDTKGDRYSSPVVPELQILGYPLPNADTIMKTVTTAKELSQQKDKFSQKMLDELKIKEMALETSLNSKIFDVTAINANAGVLKDCIEKRQLLKK

SEQ ID NO: 48 - protein, 843 aa, Streptococcus pyogenes
MDKHLLVKRTLGCVCAATLMGAALATHHDSLNTVKAEEKTVQTGKTDQQVGAKLVQEIREGKRGPLYAGYFRTWHDRASTGIDGKQQHPENTMAEVPKEVDILFVFHDHTASDSPFWSELKDSYVHKLHQQGTALVQTIGVNELNGRTGLSKDYPDTPEGNKALAAAIVKAFVTDRGVDGLDIDIEHEFTNKRTPEEDARALNVFKEIAQLIGKNGSDKSKLLIMDTTLSVENNPIFKGIAEDLDYLLRQYYGSQGGEAEVDTINSDWNQYQNYIDASQFMIGFSFFEESASKGNLWFDVNEYDPNNPEKGKDIEGTRAKKYAEWQPSTGGLKAGIFSYAIDRDGVAHVPSTYKNRTSTNLQRHEVDNISHTDYTVSRKLKTLMTEDKRYDVIDQKDIPDPALREQIIQQVGQYKGDLERYNKTLVLTGDKIQNLKGLEKLSKLQKLELRQLSNVKEITPELLPESMKKDAELVMVGMTGLEKLNLSGLNRQTLDGIDVNSITHLTSFDISHNSLDLSEKSEDRKLLMTLMEQVSNHQKITVKNTAFENQKPKGYYPQTYDTKEGHYDVDNAEHDILTDFVFGTVTKRNTFIGDEEAFAIYKEGAVDGRQYVSKDYTYEAFRKDYKGYKVHLTASNLGETVTSKVTATTDETYLVDVSDGEKVVHHMKLNIGSGAIMMENLAKGAKVIGTSGDFEQAKKIFDGEKSDRFFTWGQTNWIAFDLGEINLAKEWRLFNAETNTEIKTDSSLNVAKGRLQILKDTTIDLEKMDIKNRKEYLSNDENWTDVAQMDDAKAIFNSKLSNVLSRYWRFCVDGGASSYYPQYTELQILGQRLSNDVANTLKD

SEQ ID NO: 49 - protein, 928 aa, Streptococcus iniae
MNKRLLVKRTFGCVCAAAILGVAPLSHPTIVEAREELKMPNGLEQSIADVEAKIDALTYLSKNSKDEFKHSMYEIPSNREHKPVSPKQALQNAKKADAQAERLAKMTIPKKEELKALEGPLYGGYFRTWQDKTSDPTETNKVNSFGELPKEVDLAFVFHDYTKDYSLFWEELATKQVPKLNKQGTRVIRTIPWRFLSGADHSDISADKEKFPNTEAGNKALAKAIVDEYVYKYNLDGLDIDIERDSVPKVNDKEDPEALARTVEVFKEIGKLIGANGADKSRLLIMDTTYTAEENPLIKETAQYLNLLLVQVYGFSGENGNYLHHKNILDETSSMEGRWQGYSKYIRPEQYMVGFSFYEEKDFNNRWKDINEEDPSDPHIGEKIQGTRAERYAKWQPKTGGLKGGLFSYAIDRDGVAQPKQKTEHPELDKIVKSEYKVSKALKKLMMTDDQYQPIDQSDFPDKALRESIIKQVGTRRGDLERFKGTLRLDNPEIKDLTGLNKLKRVAKLELINLPKITKIDKDDLPQNLKPLTDNQKSNLEIKGTYDDSKLYKDIPAFDLVISGLSGLESLDISGHQRDTLSGIDASTLPSLKAINISDNHFDLAQGTENRHILDTILATLAKNGASTASFDKQKPKGLYPESYSTAPLHLQVGQGKINVIDDLIFGTRTNQNTLINTENDFEAYKEQTIQGKPFIAPDYLYDNFKVSYKEYSASIVDSTLAETTDKTIDTAKAETYQVTVSNKDGKTVHSVKVIVGDEKPMMVNLAQDAKIIGTDNMTQSAKVFDGQKDQFLLSWNKDSSVIFELKTPGTAKHWRFFDDGKNDSVTLSVFKGDASNFETEKDKAENWVEITKDSRKNDDKVFSSPLEVDNAKYLKVTIKKEAKYIYFNELQILGYPGVVAKKTADDLRPTEADKSDDKSDKNDTEAK

SEQ ID NO: 50 - protein, 744 aa, Mucor hiemalis
MPSLQLQPDDKLAPVSFALKSMNELRDWTPDEKIKFNVSSVALQPRVKNALKPQLLLTHDMAGGYKEDKNIQGNNYKDIYNIQYWHLADTFVYFSHERVSIPPVNWTNACHRNGVKCLGTFLVEGNNQMHEMEALLHGPPLLNNTDDPMRLWSPYYADQLVAIAKHYGFDGWLFNIECEFFPFPTNPKFKAEELAKFLHYFKEKLHNEIPGSQLIWYDSMTNEGEIHWQNQLTWKNELFFKNTDGIFLNYWWKKEYPEMARRVAEGIGRSGLEVYFGTDVWGRHTYGGGGFKSYKGVKTAYSAMTSSALFGMAWTYEHFEKSEFEKMDRLFWCGGKYSDYPPPPPKNPDDEKEVESDDSEDELMYGHKKGIADTVESIPVPGTDWFVTNFDRGFGNRFYYRGKRLLSQPWSHLSHQAILPNKSYRNPEIYPTDQNIKITSSLDCDHGAFLGGTSLIIKGQRFNHRESHDVETEISIPLYKLSLDASKGCSLRYIYRTLLMKDVKLTVACHFSLKTNDSVNFFKVWQPDENFSFEYDDGMRATVTTENSTESRCFLLRTTEEDTGENDWITKTINVPAVPEGSQLYITRLEVSVVLDTAGLVGLVNQVIACLGYISIIPTINSGIKTDSSRIIQDLFWKDQKYTKIGKESLDDIAQEEVHRYYGTLNWENTANVVNAWEEIDYYNVFYKESDDSATRIFLGTAFCNQFRVSGLDIILSKLPKIVIEAVNKEGYISSSGSIDLSLN

SEQ ID NO: 51 - protein, 696 aa, Rhizomucor pusillus [sequence omitted]

SEQ ID NO: 52 - protein, 787 aa, Coprinopsis cinerea
MPIAGKKFHPRALPEFWRTFREMDEWRATQTGPQARPAEGILKYVPRKIRPADIAGKGRLLVSHDYKGGYVEDPFSKSYSFNWWFSTDSFNYFAHHRITIPPPEWINAAHRQGVPILGTIIFEGGSDEDILRMVIGKTPGSTSNFHAERNAEYTVPVSSYYAELFADLAVERGFDGWLLNVEIGLQGGSEQARGLAAWVALLQQEVLKKVGPHGLVIWYDSVTVRGDLWWQDRLNAFNLPFFLNSSGIFTNYWWYNDAPQKQIDFLSRVDPNLTGQTAEPHQYNLQKTIQDIYIGVDVWGRGSHGGGGFGAYKAIEHADPKGLGFSVALFAQGWTWETEEEKPGWNWAQFWDYDSKLWVGPPGVVEAPDHTVKPGEYPCVHGPFQPISSFFLTYPPPDPLDLPFYTNFCPGIGDAWFVEGKEVFRSETGWTDMDKQTTVGDLVWPRPKIYDLPSQNASQATLNAAFNFNDAWNGGNSLQINLTVPGGATTYGAYWVPIQTFTFSSRRQYEASIVYKPGLSGKTRFDAKYEVGIRTITGEDQGKIISNTTTEVGNGWRKVHILFEIETPVEGGSIIVPSSIGLVIAVSNVSTTEQFEFPFLVGQITIHPHLPDRYKEFKPALLWLLFTPSAGTNSLDGTLTWDVVAAIERPPPVEINNPDDAQIPWNLQPTKQEWFPDFLYFNVYVLELLDGGGQGPPQWIGTTGYDGEKKRFFIYDESLPPTSGLRRFTFQIEGVLETGESTHWYDAPAAPSATAGGEQKRTRRTSLKSVLSPLRRKKSKGDISVAK

SEQ ID NO: 53 - protein, 772 aa, Ogataea minuta
MAQSQLLGGAVRPVFFDKLEELRRWHTQSANLSRESELDSLNVATEPFSSYERAQTGSGSRSSEPVPGDKEDPPIKLMVCHDFKGGYQDYEDAQPLGYFPHPTGSRYFLQYPQLIDQFVYFSHHRVTVPPVNWINFCHRNGIKCFGTVIFEGNASKDFEELDRLVSRDEKGDFVFVDALIKLAAHYGFDGYLLNIETTFSNTKIAADLEPFAEQLKSGLHCLDSKNELIWYDSYVFPANKVSYTNGVTESNYNFFSLSDAFFSNYWWNIKNLQENIKNVGVLGVQKKIYVGYDVWGRGTLVGKGGFDSSLACKMIAKFKSNVALFAPAWTYESLGPKDFNQNDARFWIGLFENESSISSTVPPHSSAVYKINESSFIFYTNFSSGEGNRFFSKGSEVYRKNWVNGSLQFDLPIDLHRKDKNGLQWALDKSDAFHGGACLEIKYSEIKDENGYQIFNNQMVSDFTLFNFTKECHFPTVNVKVTYKLNHKTKSTFKIKIKYIIERRFRSVQTVRTGYLTIPLLSTSGKWFTVEESFQINLQTSHEYIVLESAHVTYDEDRSADSFFRSYIVEDSAITSVIDNEEYEKLINSEIYNDDEDEDWILVPSDVSISSSESQSNDSKTQYLGRKLFGNKSTPKTRTLEGTAPLLRIGEFAIISANNYPSSNFLAVTSVKSIESSRLEGDSLVLLNWQVGEGHQKGVCYYIIYVNGAVVGLSVAPKFIYQDTELASENSASARSNYKKSGLGSSSDRKSKVRVDSVDKLGNVFTGSEVWV

SEQ ID NO: 54 - protein, 1067 aa, Streptococcus dysgalactiae
MDKRLLVKRTLGCVCSATLMGTILGTHHDSLISVKAEEKITQVSQTSTSIDDLHYLSENSKKEFKEELSKEKVPEKVKEILSKAQQANKQAQELAEMKVPDKIPMKPLNGPLYGGYFRTWHDKTSDPLEKDKVNSMGELPKEVDLAFVFHDWTKDYSLFWKELATKHVPKLNKQGTRVIRTIPWRFLAGGDNSGIAEDASKYPNTPEGNKALAKAIVDEYVYKYNLDGLDVDIEHDSIPKVNGEASDENLKRSIDVFEEIGKLIGPKGADKSRLFIMDSTYMADKNPLIERGAPYIDLLLVQVYGSQGEQGEFQNDTKSVTKTPEERWQGYSKYIRPEQYMIGFSFYEEKAGSGNLWYDINARKDEDTANGINDDITGTRAERYARWQPKTGGVKGGIFSYAIDRDGVAHQPKQIAEKDKQSVKNNRPLISEITDNIFHSNYSVSKTLKTVMLKDKAYDLIDEKDFPDKALREAVMAQVGTRKGDLERFNGTLRLDNPAIQSLEGLNKFKKLAQLDLIGLSRIIKLDQSVLPANMKPGKDPLETVLETYKKNGKEEPAIIPPVSLTVSGLTGLKELDLSGFDRETLAGIDAATLTSLEKVDISDNKLDLAPKTENRQIFDVMLSTVNNNAGISEQSIKFDNQKPAGNYPQTYGATNLQLPVRQEKIDLQHQLLFGTITNQGTLINSEADYKTYRNQKIAGRNFVDPDYPYNNFKVSHDNYTVKVTDSTLGTTTDKMLATDKEETYKVDFFSPTDKTKAVHTAKVIVGDEKTMMVNLAEGATVIKSENDENAQKVFNGIMEYNPLSFNNKSSIIFEIKDPSLAKYWRLFNDSSKDKKDYIKEAKLEVFTGQLNAEADVKTILEKPDNWVTVSTYSGEEKVFSHSLDNISAKYWRVTVDNKKDQYGYVSLPELQILGYPLPNADTIMKTVTVAKELSQQKDKFPQQLLDESTAKEAVVEASLNSKLFDTGVINTNVEALKNVVDECLAYEKNKETAFKATEDYRAAVNGVKAESVTVEEMAQLKDLIGKAAHLNSKIDAKLADREYDKDLLGLIGELTNITRTVKSFVK

SEQ ID NO: 55 - protein, 1011 aa, Streptococcus equi
MEKQVLVKKTLKCVCAAALMVAILAAQHDSLIRVKAEDKLVQTSPSVSAIDALHYLSENSKKEFKEELSKVEKAQPEKLKEIVSKAQQADKQAKTLAEMKVPEKIPMKPLKGPLYGGYFRTWHDKTSDPAEKDKVNSMGELPKEVDLAFVFHDWTKDYSLFWQELATKHVPTLNKQGTRVIRTIPWRFLAGGDHSGIAEDAQKYPNTPEGNKALAKAIVDEYVYKYNLDGLDVDIERDSIPKVNKEESKEGIERSIQVFEEIGKLIGPKGADKSRLFIMDSTYMADKNPLIERGAPYIDLLLVQVYGTQGEKGGFDNANHKAVDTMEERWESYSKYIRPEQYMVGFSFYEEKANSGNLWYDVNVEDDTNPNIGSEIKGTRAERYAKWQPKTGGVKGGIFSYGIDRDGVAHPKKNGPKTPDLDKIVKSDYKVSKALKKVMENDKSYELIDQKDFPDKALREAVIAQVGSRRGNLERFNGTLRLDNPDIKSLEGLNKLKKLAKLELIGLSQITKLDSSVLPENIKPTKDTLVSVLETYKNDDRKEEAKAIPQVALTISGLTGLKELNLAGFDRDSLAGIDAASLTSLEKVDLSSNKLDLAAGTENRQILDTMLATVTKHGGVSEKTFVFDHQKPTGLYPDTYGTKSLQLPVANDTIDLQAKLLFGTVTNQGTLINSEADYKAYQEQEIAGHRFVDSSYDYKAFAVTYKDYKIKVTDSTLGVTDHKDLSTSKEETYKVEFFSPINSTKPVHEAKIVVGEEKTMMVNLAEGATIIGGDADPTNAKKVFDGLLNNDTTTLSTSNKASIIFELKEPGLVKHWRFFNDSKISKADYIKEAKLEAFVGHLEDSSKVKDSLEKSTEWVTVSDYSGEAQEFSQPLNNIGAKYWRITIDNKKSQYGYVSLPELQIIGHRLPEAATVMTTMAAAEELSQQKDKFSQEQLKELEVKVAALKAALDNKMFNADTINASFADVKAYIDKLLADAAGKKTLGKATKEAQPVATDAKEKAESENPKAD

SEQ ID NO: 56 - protein, 1018 aa, Streptococcus equi
MEKQVLVKKTLKCVCAAALMVAILAAQHDSLIRVKAEDKVVQTSPSVSAIDDLHYLSENSKKEFKEGLSKAGEVPEKLKDILSKAQQADKQAKVLAEMKVPEKIAMKPLKGPLYGGYFRTWHDKTSDPAEKDKVNSMGELPKEVDLAFVFHDWTKDYSFFWQELATKHVPTLNKQGTRVIRTIPWRFLAGGDHSGIAEDTQKYPNTPEGNKALAKAIVDEYVYKYNLDGLDVDIERDSIPKVNGKESNENIQRSIAVFEEIGKLIGPKGADKSRLFIMDSTYMADKNPLIERGAQYIDLLLVQVYGTQGEKGDWDPVARKPEKTMEERWESYSKYIRPEQYMVGFSFYEENAGSGNLWYDINERKDDHNPLNSEIAGTRAERYAKWQPKTGGVKGGIFSYAIDRDGVAHQPKKVSDDEKRTNKAIKDITDGIVKSDYKVSKALKKVMENDKSYELIDQKDFPDKALREAVIAQVGSRRGDLERFNGTLRLDNPDIKSLEGLNKLKKLAKLELIGLSQITKLDSLVLPANAKPTKDTLANVLEAYDSAKKEETKAIPQVALTISGLTGLKELNLAGFDRDSLAGIDAASLTSLEKVDLSSNKLDLAAGTENRQILDTMLATVTKHGGVSEKTFVFDHQKPTGLYPDTYGTKSLQLPVANDTIDLQAKLLFGTVTNQGTLINSEADYKAYQEQEIAGHRFVDSSYDYKAFAVTYKDYKIKVTDSTLGVTDHKDLSTSKEETYKVEFFSPTNSTKPVHEAKVVVGAEKTMMVNLAEGATVIGGDADPTNAKKVFDGLLNNDTTILSTSNKASIIFELKEPGLVKYWRFFNDSKISKADCIKEAKLEAFVGHLEAGSKVKDSLEKSSKWVTVSDYSGEDQEFSQPLNNIGAKYWRITVDTKGGRYNWPSLPELQIIGYQLPAADLVMAMLATAEELSQQKDKFSQEQLKELEVKIAALKAALDSKMFNADAINASTADLKAYVDKLLADRTDQEKVAKAAKVEQPVATDIKENTEPENPKTD